European Patent Specification EP 3 983 429 B1, published April 15, 2026. Title: Amino acid sequences of recombinant flavivirus proteins and recombinant flavivirus-like particles, their use in preventing Zika virus infections, and their in vitro diagnostic application. Applicant: Uniwersytet Gdanski. The sequence listing filed with the application follows.

SEQUENCE LISTING (11 sequences)

SEQ ID NO: 1 - protein, 184 aa, Artificial Sequence
  SIGNAL 1..16: SEQ 11
  optssprM
MVGVALALALATTAMAAEVTRRGSAYYMYLDRNDAGEAISFPTTLGMNKCYIQIMDLGHMCDATMSYECPMLDEGVEPDDVDCWCNTTSTWVVYGTCHHKKGEARRSRRAVTLPSHSTRKLQTRSQTWLESREYTKHLIRVENWIFRNPGFALAAAAIAWLLGSSTSQKVIYLVMILLIAPAYS

SEQ ID NO: 2 - protein, 522 aa, Artificial Sequence
  SIGNAL 1..16: SEQ 11
  optssE
MVGVALALALATTAMAIRCIGVSNRDFVEGMSGGTWVDVVLEHGGCVTVMAQDKPTVDIELVTTTVSNMAEVRSYCYEASISDMASDSRCPTQGEAYLDKQSDTQYVCKRTLVDRGWGNGCGLFGKGSLVTCAKFACSKKMTGKSIQPENLEYRIMLSVHGSQHSGMIVNDTGHETDENRAKVEITPNSPRAEATLGGFGSLGLDCEPRTGLDFSDLYYLTMNNKHWLVHKEWFHDIPLPWHAGADTGTPHWNNKEALVEFKDAHAKRQTVVVLGSQEGAVHTALAGALEAEMDGAKGRLSSGHLKCRLKMDKLRLKGVSYSLCTAAFTFTKIPAETLHGTVTVEVQYAGTDGPCKVPAQMAVDMQTLTPVGRLITANPVITESTENSKMMLELDPPFGDSYIVIGVGEKKITHHWHRSGSTIGKAFEATVRGAKRMAVLGDTAWDFGSVGGALNSLGKGIHQIFGAAFKSLFGGMSWFSQILIGTLLMWLGLNTKNGSISLMCLALGGVLIFLSTAVSADV

SEQ ID NO: 3 - protein, 522 aa, Artificial Sequence
  ssEchimera
  DOMAIN 426..522: domeny helikalne i transmembranowe białka E wirusa TBEV
SQKVIYLVMILLIAPAYSIRCIGVSNRDFVEGMSGGTWVDVVLEHGGCVTVMAQDKPTVDIELVTTTVSNMAEVRSYCYEASISDMASDSRCPTQGEAYLDKQSDTQYVCKRTLVDRGWGNGCGLFGKGSLVTCAKFACSKKMTGKSIQPENLEYRIMLSVHGSQHSGMIVNDTGHETDENRAKVEITPNSPRAEATLGGFGSLGLDCEPRTGLDFSDLYYLTMNNKHWLVHKEWFHDIPLPWHAGADTGTPHWNNKEALVEFKDAHAKRQTVVVLGSQEGAVHTALAGALEAEMDGAKGRLSSGHLKCRLKMDKLRLKGVSYSLCTAAFTFTKIPAETLHGTVTVEVQYAGTDGPCKVPAQMAVDMQTLTPVGRLITANPVITESTENSKMMLELDPPFGDSYIVIGVGEKKITHHWHRSGSTIGRVFQKTKKGIERLTVIGEHAWDFGSAGGFLSSIGKAVHTVLGGAFNSIFGGVGFLPKLLLGVALAWLGLNMRNPTMSMSFLLAGGLVLAMTLGVGA

SEQ ID NO: 4 - protein, 520 aa, Artificial Sequence
  SIGNAL 1..16: SEQ 11
  optssEchimera
  DOMAIN 424..520: TBEV stem/anchor
MVGVALALALATTAMAIRCIGVSNRDFVEGMSGGTWVDVVLEHGGCVTVMAQDKPTVDIELVTTTVSNMAEVRSYCYEASISDMASDSRCPTQGEAYLDKQSDTQYVCKRTLVDRGWGNGCGLFGKGSLVTCAKFACSKKMTGKSIQPENLEYRIMLSVHGSQHSGMIVNDTGHETDENRAKVEITPNSPRAEATLGGFGSLGLDCEPRTGLDFSDLYYLTMNNKHWLVHKEWFHDIPLPWHAGADTGTPHWNNKEALVEFKDAHAKRQTVVVLGSQEGAVHTALAGALEAEMDGAKGRLSSGHLKCRLKMDKLRLKGVSYSLCTAAFTFTKIPAETLHGTVTVEVQYAGTDGPCKVPAQMAVDMQTLTPVGRLITANPVITESTENSKMMLELDPPFGDSYIVIGVGEKKITHHWHRSGSTIGRVFQKTKKGIERLTVIGEHAWDFGSAGGFLSSIGKAVHTVLGGAFNSIFGGVGFLPKLLLGVALAWLGLNMRNPTMSMSFLLAGGLVLAMTLGVGA

SEQ ID NO: 5 - protein, 690 aa, Artificial Sequence
  SIGNAL 1..16: SEQ 11
  optssprME
MVGVALALALATTAMAAEVTRRGSAYYMYLDRNDAGEAISFPTTLGMNKCYIQIMDLGHMCDATMSYECPMLDEGVEPDDVDCWCNTTSTWVVYGTCHHKKGEARRSRRAVTLPSHSTRKLQTRSQTWLESREYTKHLIRVENWIFRNPGFALAAAAIAWLLGSSTSQKVIYLVMILLIAPAYSIRCIGVSNRDFVEGMSGGTWVDVVLEHGGCVTVMAQDKPTVDIELVTTTVSNMAEVRSYCYEASISDMASDSRCPTQGEAYLDKQSDTQYVCKRTLVDRGWGNGCGLFGKGSLVTCAKFACSKKMTGKSIQPENLEYRIMLSVHGSQHSGMIVNDTGHETDENRAKVEITPNSPRAEATLGGFGSLGLDCEPRTGLDFSDLYYLTMNNKHWLVHKEWFHDIPLPWHAGADTGTPHWNNKEALVEFKDAHAKRQTVVVLGSQEGAVHTALAGALEAEMDGAKGRLSSGHLKCRLKMDKLRLKGVSYSLCTAAFTFTKIPAETLHGTVTVEVQYAGTDGPCKVPAQMAVDMQTLTPVGRLITANPVITESTENSKMMLELDPPFGDSYIVIGVGEKKITHHWHRSGSTIGKAFEATVRGAKRMAVLGDTAWDFGSVGGALNSLGKGIHQIFGAAFKSLFGGMSWFSQILIGTLLMWLGLNTKNGSISLMCLALGGVLIFLSTAVSADV

SEQ ID NO: 6 - protein, 688 aa, Artificial Sequence
  SIGNAL 1..16: SEQ 11
  optssprMEchimera
  DOMAIN 592..688: TBEV stem/anchor
MVGVALALALATTAMAAEVTRRGSAYYMYLDRNDAGEAISFPTTLGMNKCYIQIMDLGHMCDATMSYECPMLDEGVEPDDVDCWCNTTSTWVVYGTCHHKKGEARRSRRAVTLPSHSTRKLQTRSQTWLESREYTKHLIRVENWIFRNPGFALAAAAIAWLLGSSTSQKVIYLVMILLIAPAYSIRCIGVSNRDFVEGMSGGTWVDVVLEHGGCVTVMAQDKPTVDIELVTTTVSNMAEVRSYCYEASISDMASDSRCPTQGEAYLDKQSDTQYVCKRTLVDRGWGNGCGLFGKGSLVTCAKFACSKKMTGKSIQPENLEYRIMLSVHGSQHSGMIVNDTGHETDENRAKVEITPNSPRAEATLGGFGSLGLDCEPRTGLDFSDLYYLTMNNKHWLVHKEWFHDIPLPWHAGADTGTPHWNNKEALVEFKDAHAKRQTVVVLGSQEGAVHTALAGALEAEMDGAKGRLSSGHLKCRLKMDKLRLKGVSYSLCTAAFTFTKIPAETLHGTVTVEVQYAGTDGPCKVPAQMAVDMQTLTPVGRLITANPVITESTENSKMMLELDPPFGDSYIVIGVGEKKITHHWHRSGSTIGRVFQKTKKGIERLTVIGEHAWDFGSAGGFLSSIGKAVHTVLGGAFNSIFGGVGFLPKLLLGVALAWLGLNMRNPTMSMSFLLAGGLVLAMTLGVGA

SEQ ID NO: 7 - protein, 732 aa, Artificial Sequence
  ss1prMP2AssE
  SITE 187..189: GSG
  PEPTIDE 190..208: P2A
GADTSVGIVGLLLTTAMAAEVTRRGSAYYMYLDRNDAGEAISFPTTLGMNKCYIQIMDLGHMCDATMSYECPMLDEGVEPDDVDCWCNTTSTWVVYGTCHHKKGEARRSRRAVTLPSHSTRKLQTRSQTWLESREYTKHLIRVENWIFRNPGFALAAAAIAWLLGSSTSQKVIYLVMILLIAPAYSGSGATNFSLLKQAGDVEENPGPSQKVIYLVMILLIAPAYSIRCIGVSNRDFVEGMSGGTWVDVVLEHGGCVTVMAQDKPTVDIELVTTTVSNMAEVRSYCYEASISDMASDSRCPTQGEAYLDKQSDTQYVCKRTLVDRGWGNGCGLFGKGSLVTCAKFACSKKMTGKSIQPENLEYRIMLSVHGSQHSGMIVNDTGHETDENRAKVEITPNSPRAEATLGGFGSLGLDCEPRTGLDFSDLYYLTMNNKHWLVHKEWFHDIPLPWHAGADTGTPHWNNKEALVEFKDAHAKRQTVVVLGSQEGAVHTALAGALEAEMDGAKGRLSSGHLKCRLKMDKLRLKGVSYSLCTAAFTFTKIPAETLHGTVTVEVQYAGTDGPCKVPAQMAVDMQTLTPVGRLITANPVITESTENSKMMLELDPPFGDSYIVIGVGEKKITHHWHRSGSTIGKAFEATVRGAKRMAVLGDTAWDFGSVGGALNSLGKGIHQIFGAAFKSLFGGMSWFSQILIGTLLMWLGLNTKNGSISLMCLALGGVLIFLSTAVSADV

SEQ ID NO: 8 - protein, 730 aa, Artificial Sequence
  ss1prMP2AssEchimera
  SITE 187..189: GSG
  PEPTIDE 190..208: P2A
  DOMAIN 634..730: TBEV stem/anchor
GADTSVGIVGLLLTTAMAAEVTRRGSAYYMYLDRNDAGEAISFPTTLGMNKCYIQIMDLGHMCDATMSYECPMLDEGVEPDDVDCWCNTTSTWVVYGTCHHKKGEARRSRRAVTLPSHSTRKLQTRSQTWLESREYTKHLIRVENWIFRNPGFALAAAAIAWLLGSSTSQKVIYLVMILLIAPAYSGSGATNFSLLKQAGDVEENPGPSQKVIYLVMILLIAPAYSIRCIGVSNRDFVEGMSGGTWVDVVLEHGGCVTVMAQDKPTVDIELVTTTVSNMAEVRSYCYEASISDMASDSRCPTQGEAYLDKQSDTQYVCKRTLVDRGWGNGCGLFGKGSLVTCAKFACSKKMTGKSIQPENLEYRIMLSVHGSQHSGMIVNDTGHETDENRAKVEITPNSPRAEATLGGFGSLGLDCEPRTGLDFSDLYYLTMNNKHWLVHKEWFHDIPLPWHAGADTGTPHWNNKEALVEFKDAHAKRQTVVVLGSQEGAVHTALAGALEAEMDGAKGRLSSGHLKCRLKMDKLRLKGVSYSLCTAAFTFTKIPAETLHGTVTVEVQYAGTDGPCKVPAQMAVDMQTLTPVGRLITANPVITESTENSKMMLELDPPFGDSYIVIGVGEKKITHHWHRSGSTIGRVFQKTKKGIERLTVIGEHAWDFGSAGGFLSSIGKAVHTVLGGAFNSIFGGVGFLPKLLLGVALAWLGLNMRNPTMSMSFLLAGGLVLAMTLGVGA

SEQ ID NO: 9 - protein, 730 aa, Artificial Sequence
  SIGNAL 1..16: SEQ 11
  optssprMP2AssE
  SITE 185..187: GSG
  PEPTIDE 188..206: P2A
MVGVALALALATTAMAAEVTRRGSAYYMYLDRNDAGEAISFPTTLGMNKCYIQIMDLGHMCDATMSYECPMLDEGVEPDDVDCWCNTTSTWVVYGTCHHKKGEARRSRRAVTLPSHSTRKLQTRSQTWLESREYTKHLIRVENWIFRNPGFALAAAAIAWLLGSSTSQKVIYLVMILLIAPAYSGSGATNFSLLKQAGDVEENPGPSQKVIYLVMILLIAPAYSIRCIGVSNRDFVEGMSGGTWVDVVLEHGGCVTVMAQDKPTVDIELVTTTVSNMAEVRSYCYEASISDMASDSRCPTQGEAYLDKQSDTQYVCKRTLVDRGWGNGCGLFGKGSLVTCAKFACSKKMTGKSIQPENLEYRIMLSVHGSQHSGMIVNDTGHETDENRAKVEITPNSPRAEATLGGFGSLGLDCEPRTGLDFSDLYYLTMNNKHWLVHKEWFHDIPLPWHAGADTGTPHWNNKEALVEFKDAHAKRQTVVVLGSQEGAVHTALAGALEAEMDGAKGRLSSGHLKCRLKMDKLRLKGVSYSLCTAAFTFTKIPAETLHGTVTVEVQYAGTDGPCKVPAQMAVDMQTLTPVGRLITANPVITESTENSKMMLELDPPFGDSYIVIGVGEKKITHHWHRSGSTIGKAFEATVRGAKRMAVLGDTAWDFGSVGGALNSLGKGIHQIFGAAFKSLFGGMSWFSQILIGTLLMWLGLNTKNGSISLMCLALGGVLIFLSTAVSADV

SEQ ID NO: 10 - protein, 728 aa, Artificial Sequence
  SIGNAL 1..16: SEQ 11
  optssprMP2AssEchimera
  SITE 185..187: GSG
  PEPTIDE 188..206: P2A
  DOMAIN 632..728: TBEV stem/anchor
MVGVALALALATTAMAAEVTRRGSAYYMYLDRNDAGEAISFPTTLGMNKCYIQIMDLGHMCDATMSYECPMLDEGVEPDDVDCWCNTTSTWVVYGTCHHKKGEARRSRRAVTLPSHSTRKLQTRSQTWLESREYTKHLIRVENWIFRNPGFALAAAAIAWLLGSSTSQKVIYLVMILLIAPAYSGSGATNFSLLKQAGDVEENPGPSQKVIYLVMILLIAPAYSIRCIGVSNRDFVEGMSGGTWVDVVLEHGGCVTVMAQDKPTVDIELVTTTVSNMAEVRSYCYEASISDMASDSRCPTQGEAYLDKQSDTQYVCKRTLVDRGWGNGCGLFGKGSLVTCAKFACSKKMTGKSIQPENLEYRIMLSVHGSQHSGMIVNDTGHETDENRAKVEITPNSPRAEATLGGFGSLGLDCEPRTGLDFSDLYYLTMNNKHWLVHKEWFHDIPLPWHAGADTGTPHWNNKEALVEFKDAHAKRQTVVVLGSQEGAVHTALAGALEAEMDGAKGRLSSGHLKCRLKMDKLRLKGVSYSLCTAAFTFTKIPAETLHGTVTVEVQYAGTDGPCKVPAQMAVDMQTLTPVGRLITANPVITESTENSKMMLELDPPFGDSYIVIGVGEKKITHHWHRSGSTIGRVFQKTKKGIERLTVIGEHAWDFGSAGGFLSSIGKAVHTVLGGAFNSIFGGVGFLPKLLLGVALAWLGLNMRNPTMSMSFLLAGGLVLAMTLGVGA

SEQ ID NO: 11 - protein, 16 aa, Artificial Sequence
  SIGNAL 1..16
  optss
MVGVALALALATTAMA